European Patent Application EP 4 524 228 A1, published March 19, 2025. Title: METHOD AND DEVICE FOR DETECTING MICROORGANISM. Applicant: キッコーマン株式会社. The sequence listing filed with the application follows.

SEQUENCE LISTING (2 sequences)

SEQ ID NO: 1 - RNA, 102 nt, synthetic construct
  source 1..102: mol_type = other RNA
agaacgaatgcgaaagaagatagttttagagctagaaatagcaagttaaaataaggctagtccgttatcaacttgaaaaagtggcaccgagtcggtgctttt

SEQ ID NO: 2 - DNA, 23 bp, synthetic construct
  source 1..23: mol_type = other DNA
aacgaatgcgaaagaagatatgg